European Patent Specification EP 3 589 734 B1, published May 6, 2026. Title: REGULATION OF GENE EXPRESSION BY APTAMER-MODULATED. Applicant: MeiraGTx, LLC Guo, Xuecui. The sequence listing filed with the application follows.

SEQUENCE LISTING (16 sequences)

SEQ ID NO: 1 - DNA, 296 bp, Artificial Sequence
  Synthetic construct
cctcataaaggccaagaagggcggaaagatcgccgtgtaaggatccaagacgagctgtacaagtaaagcggccaattcggacaaaaacgagacgctggtggctggcactcctggtttccaggacggggttcaagtccctgcggtgtctataatcgcgtggatatggcacgcaagtttctaccgggcaccgtaaatgtccgactagacaccatctagagtcgacctgcaggcatgcaagcttcagctgctcgagggcccagatctaattcaccccaccagtgcaggctgcctatcag

SEQ ID NO: 2 - DNA, 305 bp, Artificial Sequence
  Synthetic construct
cctcataaaggccaagaagggcggaaagatcgccgtgtaaggatccaagacgagctgtacaagtaaagcggccgtaatgtataatcgcgtggatatggcacgcaagtttctaccgggcaccgtaaatgtccgactacattacgacgctggtggctggcactcctggtttccaggacggggttcaagtccctgcggtgtctttgcttggatcggccgcgactctagagtcgacctgcaggcatgcaagcttcagctgctcgagggcccagatctaattcaccccaccagtgcaggctgcctatcag

SEQ ID NO: 3 - DNA, 304 bp, Artificial Sequence
  Synthetic construct
cctcataaaggccaagaagggcggaaagatcgccgtgtaaggatccaagacgagctgtacaagtaaagcggcccgatcatataatcgcgtggatatggcacgcaagtttctaccgggcaccgtaaatgtccgactatggtcgacgctggtggctggcactcctggtttccaggacggggttcaagtccctgcggtgtctttgcttggatcggccgcgactctagagtcgacctgcaggcatgcaagcttcagctgctcgagggcccagatctaattcaccccaccagtgcaggctgcctatcag

SEQ ID NO: 4 - DNA, 310 bp, Artificial Sequence
  Synthetic construct
cctcataaaggccaagaagggcggaaagatcgccgtgtaaggatccaagacgagctgtacaagtaaagcggccggacaaaataatcgcgtggatatggcacgcaagtttctaccgggcaccgtaaatgtccgacttttgtccaacgagacgctggtggctggcactcctggtttccaggacggggttcaagtccctgcggtgtctttgcttggatcggccgcgactctagagtcgacctgcaggcatgcaagcttcagctgctcgagggcccagatctaattcaccccaccagtgcaggctgcctatcag

SEQ ID NO: 5 - DNA, 305 bp, Artificial Sequence
  Synthetic construct
cctcataaaggccaagaagggcggaaagatcgccgtgtaaggatccaagacgagctgtacaagtaaagaagacgtaatgtataatcgcgtggatatggcacgcaagtttctaccgggcaccgtaaatgtccgactacattacgacgctggtggctggcactcctggtttccaggacggggttcaagtccctgcggtgtctttgcttggatcggccgcgactctagagtcgacctgcaggcatgcaagcttcagctgctcgagggcccagatctaattcaccccaccagtgcaggctgcctatcag

SEQ ID NO: 6 - DNA, 498 bp, Artificial Sequence
  Synthetic construct
cctcataaaggccaagaagggcggaaagatcgccgtgtaaggatccaagacgagctgtacaagtaaagaagacgtaatgtataatcgcgtggatatggcacgcaagtttctaccgggcaccgtaaatgtccgactacattacgacgctggtggctggcactcctggtttccaggacggggttcaagtccctgcggtgtctttgcttggatcggccgcgactctagagtcgacctgcaggcatgcaagcttcagaagtaaagaagacgtaatgtataatcgcgtggatatggcacgcaagtttctaccgggcaccgtaaatgtccgactacattacgacgctggtggctggcactcctggtttccaggacggggttcaagtccctgcggtgtctttgcttggatcggccgcgactctagagtcgacctgcaggcatgcaagcttcagctgctcgagggcccagatctaattcaccccaccagtgcaggctgcctatcag

SEQ ID NO: 7 - DNA, 306 bp, Artificial Sequence
  Synthetic construct
cctcataaaggccaagaagggcggaaagatcgccgtgtaaggatccaagacgagctgtacaagtaaagaagagctaatgtataatcgcgtggatatggcacgcaagtttctaccgggcaccgtaaatgtccgactacattagcgacgctggtggctggcactcctggtttccaggacggggttcaagtccctgcggtgtctttgcttggatcggccgcgactctagagtcgacctgcaggcatgcaagcttcagctgctcgagggcccagatctaattcaccccaccagtgcaggctgcctatcag

SEQ ID NO: 8 - DNA, 307 bp, Artificial Sequence
  Synthetic construct
cctcataaaggccaagaagggcggaaagatcgccgtgtaaggatccaagacgagctgtacaagtaaagaagagctaatgtataatcgcgtggatatggcacgcaagtttctaccgggcaccgtaaatgtccgactacattagcagacgctggtggctggcactcctggtttccaggacggggttcaagtccctgcggtgtctttgcttggatcggccgcgactctagagtcgacctgcaggcatgcaagcttcagctgctcgagggcccagatctaattcaccccaccagtgcaggctgcctatcag

SEQ ID NO: 9 - DNA, 308 bp, Artificial Sequence
  Synthetic construct
cctcataaaggccaagaagggcggaaagatcgccgtgtaaggatccaagacgagctgtacaagtaaagaagagctaatgtataatcgcgtggatatggcacgcaagtttctaccgggcaccgtaaatgtccgactacattagcgagacgctggtggctggcactcctggtttccaggacggggttcaagtccctgcggtgtctttgcttggatcggccgcgactctagagtcgacctgcaggcatgcaagcttcagctgctcgagggcccagatctaattcaccccaccagtgcaggctgcctatcag

SEQ ID NO: 10 - DNA, 309 bp, Artificial Sequence
  Synthetic construct
cctcataaaggccaagaagggcggaaagatcgccgtgtaaggatccaagacgagctgtacaagtaaagaagagctaatgtataatcgcgtggatatggcacgcaagtttctaccgggcaccgtaaatgtccgactacattagccgagacgctggtggctggcactcctggtttccaggacggggttcaagtccctgcggtgtctttgcttggatcggccgcgactctagagtcgacctgcaggcatgcaagcttcagctgctcgagggcccagatctaattcaccccaccagtgcaggctgcctatcag

SEQ ID NO: 11 - DNA, 297 bp, Artificial Sequence
  Synthetic construct
cctcataaaggccaagaagggcggaaagatcgccgtgtaaggatccaagacgagctgtacaagtaaagcggccaattcggacaaaaacgagacgctggtggctggcactcctggtttccaggacggggttcaagtccctgcggtgtcttataatcgcgtggatatggcacgcaagtttctaccgggcaccgtaaatgtccgactaagacacatctagagtcgacctgcaggcatgcaagcttcagctgctcgagggcccagatctaattcaccccaccagtgcaggctgcctatcag

SEQ ID NO: 12 - DNA, 298 bp, Artificial Sequence
  Synthetic construct
cctcataaaggccaagaagggcggaaagatcgccgtgtaaggatccaagacgagctgtacaagtaaagcggccaattcggacaaaaacgagacgctggtggctggcactcctggtttccaggacggggttcaagtccctgcggtgtctgtataatcgcgtggatatggcacgcaagtttctaccgggcaccgtaaatgtccgactacagacaatctagagtcgacctgcaggcatgcaagcttcagctgctcgagggcccagatctaattcaccccaccagtgcaggctgcctatcag

SEQ ID NO: 13 - DNA, 299 bp, Artificial Sequence
  Synthetic construct
cctcataaaggccaagaagggcggaaagatcgccgtgtaaggatccaagacgagctgtacaagtaaagcggccaattcggacaaaaacgagacgctggtggctggcactcctggtttccaggacggggttcaagtccctgcggtgtctagtataatcgcgtggatatggcacgcaagtttctaccgggcaccgtaaatgtccgactactagacttctagagtcgacctgcaggcatgcaagcttcagctgctcgagggcccagatctaattcaccccaccagtgcaggctgcctatcag

SEQ ID NO: 14 - DNA, 314 bp, Artificial Sequence
  Synthetic construct
cctcataaaggccaagaagggcggaaagatcgccgtgtaaggatccaagacgagctgtacaagtaaagaagactgcgacgataatcgcgtggatatggcacgcaagtttctaccgggcaccgtaaatgtccgactcgtcgcagggccagtggcgcaatggataacgcgtctgactacggatcagaagattccaggttcgactcctggctggctcggtgtaggccgcgactctagagtcgacctgcaggcatgcaagcttcagctgctcgagggcccagatctaattcaccccaccagtgcaggctgcctatcag

SEQ ID NO: 15 - DNA, 307 bp, Artificial Sequence
  Synthetic construct
cctcataaaggccaagaagggcggaaagatcgccgtgtaaggatccaagacgagctgtacaagtaaagcggccgtaatgttataacctcaataatatggtttgagggtgtctaccaggaaccgtaaaatcctgattaacattacgacgctggtggctggcactcctggtttccaggacggggttcaagtccctgcggtgtctttgcttggatcggccgcgactctagagtcgacctgcaggcatgcaagcttcagctgctcgagggcccagatctaattcaccccaccagtgcaggctgcctatcag

SEQ ID NO: 16 - DNA, 275 bp, Artificial Sequence
  Synthetic construct
cctcataaaggccaagaagggcggaaagatcgccgtgtaaggatccaagacgagctgtacaagtaaagcggcctaatgtgataccagccgaaaggcccttggcagcacattagacgctggtggctggcactcctggtttccaggacggggttcaagtccctgcggtgtctttgcttggatcggccgcgactctagagtcgacctgcaggcatgcaagcttcagctgctcgagggcccagatctaattcaccccaccagtgcaggctgcctatcag